European Patent Application EP 4 527 407 A1, published March 26, 2025. Title: Antibody against mesothelin and the use thereof. Applicant: UCI Therapeutics Inc. The sequence listing filed with the application follows.

SEQUENCE LISTING (123 sequences)

SEQ ID NO: 1 - protein, 622 aa, Homo sapiens
MALPTARPLLGSCGTPALGSLLFLLFSLGWVQPSRTLAGETGQEAAPLDGVLANPPNISSLSPRQLLGFPCAEVSGLSTERVRELAVALAQKNVKLSTEQLRCLAHRLSEPPEDLDALPLDLLLFLNPDAFSGPQACTRFFSRITKANVDLLPRGAPERQRLLPAALACWGVRGSLLSEADVRALGGLACDLPGRFVAESAEVLLPRLVSCPGPLDQDQQEAARAALQGGGPPYGPPSTWSVSTMDALRGLLPVLGQPIIRSIPQGIVAAWRQRSSRDPSWRQPERTILRPRFRREVEKTACPSGKKAPEIDESLIFYKKWELEACVDAALLATQMDRVNAIPFTYEQLDVLKHKLDELYPQGYPESVIQHLGYLFLKMSPEDIRKWNVTSLETLKALLEVNKGHEMSPQVATLIDRFVKGRGQLDKDTLDTLTAFYPGYLCSLSPEELSSVPPSSIWAVRPQDLDTCDPRQLDVLYPKARLAFQNMNGSEYFVKIQSFLGGAPTEDLKALSQQNVSMDLATFMKLRTDAVLPLTVAEVQKLLGPHVEGLKAEERHRPVRDWILRQRQDDLDTLGLGLQGGIPNGYLVLDLSMQEALSGTPCLLGPGPVLTVLALLLASTLA

SEQ ID NO: 2 - protein, 25 aa, synthetic construct
QVQLQQSGPELVKPGASVKISCKAS

SEQ ID NO: 3 - protein, 8 aa, synthetic construct
GYSFTDYN

SEQ ID NO: 4 - protein, 17 aa, synthetic construct
MNWVKQSNGKSLEWIGV

SEQ ID NO: 5 - protein, 8 aa, synthetic construct
INPNYGTT

SEQ ID NO: 6 - protein, 38 aa, synthetic construct
SYNQKFKGKATITADTSSNTAYLQLSSLTSEDSAVYYC

SEQ ID NO: 7 - protein, 12 aa, synthetic construct
AKGDYDGAGFAY

SEQ ID NO: 8 - protein, 11 aa, synthetic construct
WGQGTLVTVSA

SEQ ID NO: 9 - protein, 26 aa, synthetic construct
DIVITQSPAIMSASPGEKVTMTCSAS

SEQ ID NO: 10 - protein, 5 aa, synthetic construct
SSVSY

SEQ ID NO: 11 - protein, 17 aa, synthetic construct
MHWYQQKSGTSPKRWIY

SEQ ID NO: 12 - skipped

SEQ ID NO: 13 - protein, 36 aa, synthetic construct
KLASGVPARFSGSGSGTSYSLTISSMEAEDAATYYC

SEQ ID NO: 14 - protein, 9 aa, synthetic construct
QQWSSNPLT

SEQ ID NO: 15 - protein, 11 aa, synthetic construct
FGAGTKLEIKR

SEQ ID NO: 16 - protein, 25 aa, synthetic construct
QVQLQQPGAELVKPGASVKLSCKAS

SEQ ID NO: 17 - protein, 8 aa, synthetic construct
GYTFTSYW

SEQ ID NO: 18 - protein, 17 aa, synthetic construct
MHWVKQRPGQGLEWIGM

SEQ ID NO: 19 - protein, 8 aa, synthetic construct
IHPNSGGT

SEQ ID NO: 20 - protein, 38 aa, synthetic construct
NYNEKFKSKATLTVDKSSSTAYMQLSSLTSEDSAVYYC

SEQ ID NO: 21 - protein, 14 aa, synthetic construct
ARYYYGNYVWYFDV

SEQ ID NO: 22 - protein, 11 aa, synthetic construct
WGTGTTVTVSA

SEQ ID NO: 23 - protein, 26 aa, synthetic construct
DIVLTQSPAIMSTSPGEKVTMTCTAS

SEQ ID NO: 24 - protein, 17 aa, synthetic construct
MHWYQQKSGTSPKRWIY

SEQ ID NO: 25 - protein, 36 aa, synthetic construct
KLASGVPARFSGSGSGTSYSLTISRMEAEDAATYYC

SEQ ID NO: 26 - protein, 9 aa, synthetic construct
QQWSSYPLT

SEQ ID NO: 27 - protein, 11 aa, synthetic construct
FGAGTKLEMKR

SEQ ID NO: 28 - protein, 25 aa, synthetic construct [sequence omitted]

SEQ ID NO: 29 - protein, 8 aa, synthetic construct
GYTFTDYN

SEQ ID NO: 30 - protein, 17 aa, synthetic construct
MNWVRQAPGQGLEWMGV

SEQ ID NO: 31 - protein, 38 aa, synthetic construct
SYNQKFKGRVTMTRDTSTSTVYMELSSLRSEDTAVYYC

SEQ ID NO: 32 - protein, 12 aa, synthetic construct
ARGDYDGAGFAY

SEQ ID NO: 33 - protein, 11 aa, synthetic construct
WGQGTLVTVSS

SEQ ID NO: 34 - protein, 26 aa, synthetic construct
EIVLTQSPATLSLSPGERATLSCSAS

SEQ ID NO: 35 - protein, 17 aa, synthetic construct
MHWYQQKPGQAPRLLIY

SEQ ID NO: 36 - protein, 36 aa, synthetic construct
KLASGIPARFSGSGSGTDFTLTISSLEPEDFAVYYC

SEQ ID NO: 37 - protein, 11 aa, synthetic construct
FGQGTKLEIKR

SEQ ID NO: 38 - protein, 119 aa, synthetic construct
QVQLQQSGPELVKPGASVKISCKASGYSFTDYNMNWVKQSNGKSLEWIGVINPNYGTTSYNQKFKGKATITADTSSNTAYLQLSSLTSEDSAVYYCAKGDYDGAGFAYWGQGTLVTVSA

SEQ ID NO: 39 - protein, 107 aa, synthetic construct
DIVITQSPAIMSASPGEKVTMTCSASSSVSYMHWYQQKSGTSPKRWIYDTSKLASGVPARFSGSGSGTSYSLTISSMEAEDAATYYCQQWSSNPLTFGAGTKLEIKR

SEQ ID NO: 40 - DNA, 357 bp, synthetic construct
  source 1..357: mol_type = other DNA
caggtccaactgcagcagtctggacctgagctggtgaagcctggcgcttcagtgaagatatcctgcaaggcttctggttactcattcactgactacaacatgaactgggtgaagcagagcaatggaaagagccttgagtggattggagtaattaatcctaactatggtactactagctacaatcagaagttcaagggcaaggccactataacagcagacacatcctccaacacagcctacctgcagctcagcagcctgacatctgaggactctgcagtctattactgtgcaaagggtgattacgacggggccgggtttgcttactggggccaagggactctggtcactgtctctgcg

SEQ ID NO: 41 - protein, 321 aa, synthetic construct
GATATTGTGATAACCCAGTCTCCAGCAATCATGTCTGCATCTCCAGGGGAGAAGGTCACCATGACCTGCAGTGCCAGCTCAAGTGTAAGTTACATGCACTGGTACCAGCAGAAGTCAGGCACCTCCCCCAAAAGATGGATTTATGACACATCCAAACTGGCTTCTGGAGTCCCTGCTCGCTTCAGTGGCAGTGGGTCTGGGACCTCTTACTCTCTCACAATCAGCAGCATGGAGGCTGAAGATGCTGCCACTTATTACTGCCAGCAGTGGAGTAGTAACCCACTCACGTTCGGTGCTGGGACCAAGCTGGAAATCAAACGC

SEQ ID NO: 42 - protein, 121 aa, synthetic construct
QVQLQQPGAELVKPGASVKLSCKASGYTFTSYWMHWVKQRPGQGLEWIGMIHPNSGGTNYNEKFKSKATLTVDKSSSTAYMQLSSLTSEDSAVYYCARYYYGNYVWYFDVWGTGTTVTVSA

SEQ ID NO: 43 - protein, 107 aa, synthetic construct
DIVLTQSPAIMSTSPGEKVTMTCTASSSVSYMHWYQQKSGTSPKRWIYDTSKLASGVPARFSGSGSGTSYSLTISRMEAEDAATYYCQQWSSYPLTFGAGTKLEMKR

SEQ ID NO: 44 - DNA, 363 bp, synthetic construct
  source 1..363: mol_type = other DNA
caggtccaactgcagcagcctggggctgaactggtgaagcctggggcttcagtgaagctgtcctgcaaggcttctggctacaccttcaccagctactggatgcactgggtgaagcagaggcctggacaaggccttgagtggattggaatgattcatcctaatagtggtggtactaactacaatgagaagttcaagagcaaggccacactgactgtagacaaatcctccagcacagcctacatgcaactcagcagcctgacatctgaggactctgcggtctattactgtgcaagatactactatggtaactacgtgtggtacttcgatgtctggggcacagggaccacggtcaccgtctctgcg

SEQ ID NO: 45 - DNA, 321 bp, synthetic construct
  source 1..321: mol_type = other DNA
gacattgttctcacccagtctccagcaatcatgtctacatctccgggggagaaggtcaccatgacctgcactgccagctcaagtgtaagttacatgcactggtaccagcagaagtcaggcacctcccccaaaagatggatttatgacacatccaaactggcttctggagtccctgctcgcttcagtggcagtgggtctgggacctcttactctctcacaatcagccgaatggaggctgaagatgctgccacttattactgccagcagtggagtagttacccactcacgttcggtgctgggaccaagctggaaatgaaacgc

SEQ ID NO: 46 - protein, 119 aa, synthetic construct
QVQLVQSGAEVKKPGASVKVSCKASGYTFTDYNMNWVRQAPGQGLEWMGVINPNYGTTSYNQKFKGRVTMTRDTSTSTVYMELSSLRSEDTAVYYCARGDYDGAGFAYWGQGTLVTVSS

SEQ ID NO: 47 - protein, 107 aa, synthetic construct
EIVLTQSPATLSLSPGERATLSCSASSSVSYMHWYQQKPGQAPRLLIYDTSKLASGIPARFSGSGSGTDFTLTISSLEPEDFAVYYCQQWSSNPLTFGQGTKLEIKR

SEQ ID NO: 48 - DNA, 357 bp, synthetic construct
  source 1..357: mol_type = other DNA
caggtccaactggttcagtctggagctgaggtaaagaagcctggcgcttcagtgaaggtttcctgcaaggcttctggttacaccttcactgactacaacatgaactgggtgcgacaggctcccggacaaggacttgagtggatgggagtaattaatcctaactatggtactactagctacaatcagaagttcaagggcagggtgactatgacacgcgacacatccacctctacagtgtacatggagctcagcagcctgcgctctgaggacacggcagtctattactgtgcaagaggtgattacgacggggccgggtttgcttactggggccaagggactctggtcactgtctctagc

SEQ ID NO: 49 - DNA, 321 bp, synthetic construct
  source 1..321: mol_type = other DNA
gaaattgtcttaacccagtctccagcaaccctttctttgtctccaggggagcgagcaaccctgagttgcagtgccagctcaagtgtaagttacatgcactggtaccagcagaagcctggccaagcgccccgccttctcatttatgacacatccaaactggcttctggaatacctgctcgcttcagtggcagtgggtctgggaccgactttactctcacaatcagcagcttggagccagaagattttgccgtatattactgccagcagtggagtagtaacccactcacgttcggtcaggggaccaagctggaaatcaaacgc

SEQ ID NO: 50 - protein, 15 aa, synthetic construct
GGGGSGGGGSGGGGS

SEQ ID NO: 51 - protein, 241 aa, synthetic construct
DIVITQSPAIMSASPGEKVTMTCSASSSVSYMHWYQQKSGTSPKRWIYDTSKLASGVPARFSGSGSGTSYSLTISSMEAEDAATYYCQQWSSNPLTFGAGTKLEIKRGGGGSGGGGSGGGGSQVQLQQSGPELVKPGASVKISCKASGYSFTDYNMNWVKQSNGKSLEWIGVINPNYGTTSYNQKFKGKATITADTSSNTAYLQLSSLTSEDSAVYYCAKGDYDGAGFAYWGQGTLVTVSA

SEQ ID NO: 52 - DNA, 723 bp, synthetic construct
  source 1..723: mol_type = other DNA
gatattgtgataacccagtctccagcaatcatgtctgcatctccaggggagaaggtcaccatgacctgcagtgccagctcaagtgtaagttacatgcactggtaccagcagaagtcaggcacctcccccaaaagatggatttatgacacatccaaactggcttctggagtccctgctcgcttcagtggcagtgggtctgggacctcttactctctcacaatcagcagcatggaggctgaagatgctgccacttattactgccagcagtggagtagtaacccactcacgttcggtgctgggaccaagctggaaatcaaacgcggaggtgggggcagtggaggcggtggtagtggaggcggaggaagtcaggtccaactgcagcagtctggacctgagctggtgaagcctggcgcttcagtgaagatatcctgcaaggcttctggttactcattcactgactacaacatgaactgggtgaagcagagcaatggaaagagccttgagtggattggagtaattaatcctaactatggtactactagctacaatcagaagttcaagggcaaggccactataacagcagacacatcctccaacacagcctacctgcagctcagcagcctgacatctgaggactctgcagtctattactgtgcaaagggtgattacgacggggccgggtttgcttactggggccaagggactctggtcactgtctctgcg

SEQ ID NO: 53 - protein, 243 aa, synthetic construct
DIVLTQSPAIMSTSPGEKVTMTCTASSSVSYMHWYQQKSGTSPKRWIYDTSKLASGVPARFSGSGSGTSYSLTISRMEAEDAATYYCQQWSSYPLTFGAGTKLEMKRGGGGSGGGGSGGGGSQVQLQQPGAELVKPGASVKLSCKASGYTFTSYWMHWVKQRPGQGLEWIGMIHPNSGGTNYNEKFKSKATLTVDKSSSTAYMQLSSLTSEDSAVYYCARYYYGNYVWYFDVWGTGTTVTVSA

SEQ ID NO: 54 - DNA, 729 bp, synthetic construct
  source 1..729: mol_type = other DNA
gacattgttctcacccagtctccagcaatcatgtctacatctccgggggagaaggtcaccatgacctgcactgccagctcaagtgtaagttacatgcactggtaccagcagaagtcaggcacctcccccaaaagatggatttatgacacatccaaactggcttctggagtccctgctcgcttcagtggcagtgggtctgggacctcttactctctcacaatcagccgaatggaggctgaagatgctgccacttattactgccagcagtggagtagttacccactcacgttcggtgctgggaccaagctggaaatgaaacgcggaggtgggggcagtggaggcggtggtagtggaggcggaggaagtcaggtccaactgcagcagcctggggctgaactggtgaagcctggggcttcagtgaagctgtcctgcaaggcttctggctacaccttcaccagctactggatgcactgggtgaagcagaggcctggacaaggccttgagtggattggaatgattcatcctaatagtggtggtactaactacaatgagaagttcaagagcaaggccacactgactgtagacaaatcctccagcacagcctacatgcaactcagcagcctgacatctgaggactctgcggtctattactgtgcaagatactactatggtaactacgtgtggtacttcgatgtctggggcacagggaccacggtcaccgtctctgcg

SEQ ID NO: 55 - protein, 241 aa, synthetic construct
EIVLTQSPATLSLSPGERATLSCSASSSVSYMHWYQQKPGQAPRLLIYDTSKLASGIPARFSGSGSGTDFTLTISSLEPEDFAVYYCQQWSSNPLTFGQGTKLEIKRGGGGSGGGGSGGGGSQVQLVQSGAEVKKPGASVKVSCKASGYTFTDYNMNWVRQAPGQGLEWMGVINPNYGTTSYNQKFKGRVTMTRDTSTSTVYMELSSLRSEDTAVYYCARGDYDGAGFAYWGQGTLVTVSS

SEQ ID NO: 56 - DNA, 723 bp, synthetic construct
  source 1..723: mol_type = other DNA
gaaattgtcttaacccagtctccagcaaccctttctttgtctccaggggagcgagcaaccctgagttgcagtgccagctcaagtgtaagttacatgcactggtaccagcagaagcctggccaagcgccccgccttctcatttatgacacatccaaactggcttctggaatacctgctcgcttcagtggcagtgggtctgggaccgactttactctcacaatcagcagcttggagccagaagattttgccgtatattactgccagcagtggagtagtaacccactcacgttcggtcaggggaccaagctggaaatcaaacgcggaggtgggggcagtggaggcggtggtagtggaggcggaggaagtcaggtccaactggttcagtctggagctgaggtaaagaagcctggcgcttcagtgaaggtttcctgcaaggcttctggttacaccttcactgactacaacatgaactgggtgcgacaggctcccggacaaggacttgagtggatgggagtaattaatcctaactatggtactactagctacaatcagaagttcaagggcagggtgactatgacacgcgacacatccacctctacagtgtacatggagctcagcagcctgcgctctgaggacacggcagtctattactgtgcaagaggtgattacgacggggccgggtttgcttactggggccaagggactctggtcactgtctctagc

SEQ ID NO: 57 - protein, 21 aa, synthetic construct
MALPVTALLLPLALLLHAARP

SEQ ID NO: 58 - DNA, 63 bp, synthetic construct
  source 1..63: mol_type = other DNA
atggccttaccagtgaccgccttgctcctgccgctggccttgctgctccacgccgccaggccg

SEQ ID NO: 59 - protein, 45 aa, synthetic construct
TTTPAPRPPTPAPTIASQPLSLRPEACRPAAGGAVHTRGLDFACD

SEQ ID NO: 60 - DNA, 135 bp, synthetic construct
  source 1..135: mol_type = other DNA
accacgacgccagcgccgcgaccaccaacaccggcgcccaccatcgcgtcgcagcccctgtccctgcgcccagaggcgtgccggccagcggcggggggcgcagtgcacacgagggggctggacttcgcctgtgat

SEQ ID NO: 61 - protein, 24 aa, synthetic construct
IYIWAPLAGTCGVLLLSLVITLYC

SEQ ID NO: 62 - DNA, 72 bp, synthetic construct
  source 1..72: mol_type = other DNA
atctacatctgggcgcccttggccgggacttgtggggtccttctcctgtcactggttatcaccctttactgc

SEQ ID NO: 63 - protein, 42 aa, synthetic construct
KRGRKKLLYIFKQPFMRPVQTTQEEDGCSCRFPEEEEGGCEL

SEQ ID NO: 64 - DNA, 126 bp, synthetic construct
  source 1..126: mol_type = other DNA
aaacggggcagaaagaaactcctgtatatattcaaacaaccatttatgagaccagtacaaactactcaagaggaagatggctgtagctgccgatttccagaagaagaagaaggaggatgtgaactg

SEQ ID NO: 65 - protein, 112 aa, synthetic construct
RVKFSRSADAPAYKQGQNQLYNELNLGRREEYDVLDKRRGRDPEMGGKPRRKNPQEGLYNELQKDKMAEAYSEIGMKGERRRGKGHDGLYQGLSTATKDTYDALHMQALPPR

SEQ ID NO: 66 - DNA, 336 bp, synthetic construct
  source 1..336: mol_type = other DNA
agagtgaagttcagcaggagcgcagacgcccccgcgtacaagcagggccagaaccagctctataacgagctcaatctaggacgaagagaggagtacgatgttttggacaagagacgtggccgggaccctgagatggggggaaagccgagaaggaagaaccctcaggaaggcctgtacaatgaactgcagaaagataagatggcggaggcctacagtgagattgggatgaaaggcgagcgccggaggggcaaggggcacgatggcctttaccagggtctcagtacagccaccaaggacacctacgacgcccttcacatgcaggccctgccccctcgc

SEQ ID NO: 67 - DNA, 212 bp, synthetic construct
  source 1..212: mol_type = other DNA
gggcagagcgcacatcgcccacagtccccgagaagttggggggaggggtcggcaattgatccggtgcctagagaaggtggcgcggggtaaactgggaaagtgatgtcgtgtactggctccgcctttttcccgagggtgggggagaaccgtatataagtgcagtagtcgccgtgaacgttctttttcgcaacgggtttgccgccagaacacag

SEQ ID NO: 68 - protein, 464 aa, synthetic construct
DIVITQSPAIMSASPGEKVTMTCSASSSVSYMHWYQQKSGTSPKRWIYDTSKLASGVPARFSGSGSGTSYSLTISSMEAEDAATYYCQQWSSNPLTFGAGTKLEIKRGGGGSGGGGSGGGGSQVQLQQSGPELVKPGASVKISCKASGYSFTDYNMNWVKQSNGKSLEWIGVINPNYGTTSYNQKFKGKATITADTSSNTAYLQLSSLTSEDSAVYYCAKGDYDGAGFAYWGQGTLVTVSATTTPAPRPPTPAPTIASQPLSLRPEACRPAAGGAVHTRGLDFACDIYIWAPLAGTCGVLLLSLVITLYCKRGRKKLLYIFKQPFMRPVQTTQEEDGCSCRFPEEEEGGCELRVKFSRSADAPAYKQGQNQLYNELNLGRREEYDVLDKRRGRDPEMGGKPRRKNPQEGLYNELQKDKMAEAYSEIGMKGERRRGKGHDGLYQGLSTATKDTYDALHMQALPPR

SEQ ID NO: 69 - DNA, 1392 bp, synthetic construct
  source 1..1392: mol_type = other DNA
gatattgtgataacccagtctccagcaatcatgtctgcatctccaggggagaaggtcaccatgacctgcagtgccagctcaagtgtaagttacatgcactggtaccagcagaagtcaggcacctcccccaaaagatggatttatgacacatccaaactggcttctggagtccctgctcgcttcagtggcagtgggtctgggacctcttactctctcacaatcagcagcatggaggctgaagatgctgccacttattactgccagcagtggagtagtaacccactcacgttcggtgctgggaccaagctggaaatcaaacgcggaggtgggggcagtggaggcggtggtagtggaggcggaggaagtcaggtccaactgcagcagtctggacctgagctggtgaagcctggcgcttcagtgaagatatcctgcaaggcttctggttactcattcactgactacaacatgaactgggtgaagcagagcaatggaaagagccttgagtggattggagtaattaatcctaactatggtactactagctacaatcagaagttcaagggcaaggccactataacagcagacacatcctccaacacagcctacctgcagctcagcagcctgacatctgaggactctgcagtctattactgtgcaaagggtgattacgacggggccgggtttgcttactggggccaagggactctggtcactgtctctgcgaccacgacgccagcgccgcgaccaccaacaccggcgcccaccatcgcgtcgcagcccctgtccctgcgcccagaggcgtgccggccagcggcggggggcgcagtgcacacgagggggctggacttcgcctgtgatatctacatctgggcgcccttggccgggacttgtggggtccttctcctgtcactggttatcaccctttactgcaaacggggcagaaagaaactcctgtatatattcaaacaaccatttatgagaccagtacaaactactcaagaggaagatggctgtagctgccgatttccagaagaagaagaaggaggatgtgaactgagagtgaagttcagcaggagcgcagacgcccccgcgtacaagcagggccagaaccagctctataacgagctcaatctaggacgaagagaggagtacgatgttttggacaagagacgtggccgggaccctgagatggggggaaagccgagaaggaagaaccctcaggaaggcctgtacaatgaactgcagaaagataagatggcggaggcctacagtgagattgggatgaaaggcgagcgccggaggggcaaggggcacgatggcctttaccagggtctcagtacagccaccaaggacacctacgacgcccttcacatgcaggccctgccccctcgc

SEQ ID NO: 70 - protein, 466 aa, synthetic construct
DIVLTQSPAIMSTSPGEKVTMTCTASSSVSYMHWYQQKSGTSPKRWIYDTSKLASGVPARFSGSGSGTSYSLTISRMEAEDAATYYCQQWSSYPLTFGAGTKLEMKRGGGGSGGGGSGGGGSQVQLQQPGAELVKPGASVKLSCKASGYTFTSYWMHWVKQRPGQGLEWIGMIHPNSGGTNYNEKFKSKATLTVDKSSSTAYMQLSSLTSEDSAVYYCARYYYGNYVWYFDVWGTGTTVTVSATTTPAPRPPTPAPTIASQPLSLRPEACRPAAGGAVHTRGLDFACDIYIWAPLAGTCGVLLLSLVITLYCKRGRKKLLYIFKQPFMRPVQTTQEEDGCSCRFPEEEEGGCELRVKFSRSADAPAYKQGQNQLYNELNLGRREEYDVLDKRRGRDPEMGGKPRRKNPQEGLYNELQKDKMAEAYSEIGMKGERRRGKGHDGLYQGLSTATKDTYDALHMQALPPR

SEQ ID NO: 71 - DNA, 1398 bp, synthetic construct
  source 1..1398: mol_type = other DNA
gacattgttctcacccagtctccagcaatcatgtctacatctccgggggagaaggtcaccatgacctgcactgccagctcaagtgtaagttacatgcactggtaccagcagaagtcaggcacctcccccaaaagatggatttatgacacatccaaactggcttctggagtccctgctcgcttcagtggcagtgggtctgggacctcttactctctcacaatcagccgaatggaggctgaagatgctgccacttattactgccagcagtggagtagttacccactcacgttcggtgctgggaccaagctggaaatgaaacgcggaggtgggggcagtggaggcggtggtagtggaggcggaggaagtcaggtccaactgcagcagcctggggctgaactggtgaagcctggggcttcagtgaagctgtcctgcaaggcttctggctacaccttcaccagctactggatgcactgggtgaagcagaggcctggacaaggccttgagtggattggaatgattcatcctaatagtggtggtactaactacaatgagaagttcaagagcaaggccacactgactgtagacaaatcctccagcacagcctacatgcaactcagcagcctgacatctgaggactctgcggtctattactgtgcaagatactactatggtaactacgtgtggtacttcgatgtctggggcacagggaccacggtcaccgtctctgcgaccacgacgccagcgccgcgaccaccaacaccggcgcccaccatcgcgtcgcagcccctgtccctgcgcccagaggcgtgccggccagcggcggggggcgcagtgcacacgagggggctggacttcgcctgtgatatctacatctgggcgcccttggccgggacttgtggggtccttctcctgtcactggttatcaccctttactgcaaacggggcagaaagaaactcctgtatatattcaaacaaccatttatgagaccagtacaaactactcaagaggaagatggctgtagctgccgatttccagaagaagaagaaggaggatgtgaactgagagtgaagttcagcaggagcgcagacgcccccgcgtacaagcagggccagaaccagctctataacgagctcaatctaggacgaagagaggagtacgatgttttggacaagagacgtggccgggaccctgagatggggggaaagccgagaaggaagaaccctcaggaaggcctgtacaatgaactgcagaaagataagatggcggaggcctacagtgagattgggatgaaaggcgagcgccggaggggcaaggggcacgatggcctttaccagggtctcagtacagccaccaaggacacctacgacgcccttcacatgcaggccctgccccctcgc

SEQ ID NO: 72 - protein, 464 aa, synthetic construct
EIVLTQSPATLSLSPGERATLSCSASSSVSYMHWYQQKPGQAPRLLIYDTSKLASGIPARFSGSGSGTDFTLTISSLEPEDFAVYYCQQWSSNPLTFGQGTKLEIKRGGGGSGGGGSGGGGSQVQLVQSGAEVKKPGASVKVSCKASGYTFTDYNMNWVRQAPGQGLEWMGVINPNYGTTSYNQKFKGRVTMTRDTSTSTVYMELSSLRSEDTAVYYCARGDYDGAGFAYWGQGTLVTVSSTTTPAPRPPTPAPTIASQPLSLRPEACRPAAGGAVHTRGLDFACDIYIWAPLAGTCGVLLLSLVITLYCKRGRKKLLYIFKQPFMRPVQTTQEEDGCSCRFPEEEEGGCELRVKFSRSADAPAYKQGQNQLYNELNLGRREEYDVLDKRRGRDPEMGGKPRRKNPQEGLYNELQKDKMAEAYSEIGMKGERRRGKGHDGLYQGLSTATKDTYDALHMQALPPR

SEQ ID NO: 73 - DNA, 1392 bp, synthetic construct
  source 1..1392: mol_type = other DNA
gaaattgtcttaacccagtctccagcaaccctttctttgtctccaggggagcgagcaaccctgagttgcagtgccagctcaagtgtaagttacatgcactggtaccagcagaagcctggccaagcgccccgccttctcatttatgacacatccaaactggcttctggaatacctgctcgcttcagtggcagtgggtctgggaccgactttactctcacaatcagcagcttggagccagaagattttgccgtatattactgccagcagtggagtagtaacccactcacgttcggtcaggggaccaagctggaaatcaaacgcggaggtgggggcagtggaggcggtggtagtggaggcggaggaagtcaggtccaactggttcagtctggagctgaggtaaagaagcctggcgcttcagtgaaggtttcctgcaaggcttctggttacaccttcactgactacaacatgaactgggtgcgacaggctcccggacaaggacttgagtggatgggagtaattaatcctaactatggtactactagctacaatcagaagttcaagggcagggtgactatgacacgcgacacatccacctctacagtgtacatggagctcagcagcctgcgctctgaggacacggcagtctattactgtgcaagaggtgattacgacggggccgggtttgcttactggggccaagggactctggtcactgtctctagcaccacgacgccagcgccgcgaccaccaacaccggcgcccaccatcgcgtcgcagcccctgtccctgcgcccagaggcgtgccggccagcggcggggggcgcagtgcacacgagggggctggacttcgcctgtgatatctacatctgggcgcccttggccgggacttgtggggtccttctcctgtcactggttatcaccctttactgcaaacggggcagaaagaaactcctgtatatattcaaacaaccatttatgagaccagtacaaactactcaagaggaagatggctgtagctgccgatttccagaagaagaagaaggaggatgtgaactgagagtgaagttcagcaggagcgcagacgcccccgcgtacaagcagggccagaaccagctctataacgagctcaatctaggacgaagagaggagtacgatgttttggacaagagacgtggccgggaccctgagatggggggaaagccgagaaggaagaaccctcaggaaggcctgtacaatgaactgcagaaagataagatggcggaggcctacagtgagattgggatgaaaggcgagcgccggaggggcaaggggcacgatggcctttaccagggtctcagtacagccaccaaggacacctacgacgcccttcacatgcaggccctgccccctcgc

SEQ ID NO: 74 - protein, 485 aa, synthetic construct
MALPVTALLLPLALLLHAARPDIVITQSPAIMSASPGEKVTMTCSASSSVSYMHWYQQKSGTSPKRWIYDTSKLASGVPARFSGSGSGTSYSLTISSMEAEDAATYYCQQWSSNPLTFGAGTKLEIKRGGGGSGGGGSGGGGSQVQLQQSGPELVKPGASVKISCKASGYSFTDYNMNWVKQSNGKSLEWIGVINPNYGTTSYNQKFKGKATITADTSSNTAYLQLSSLTSEDSAVYYCAKGDYDGAGFAYWGQGTLVTVSATTTPAPRPPTPAPTIASQPLSLRPEACRPAAGGAVHTRGLDFACDIYIWAPLAGTCGVLLLSLVITLYCKRGRKKLLYIFKQPFMRPVQTTQEEDGCSCRFPEEEEGGCELRVKFSRSADAPAYKQGQNQLYNELNLGRREEYDVLDKRRGRDPEMGGKPRRKNPQEGLYNELQKDKMAEAYSEIGMKGERRRGKGHDGLYQGLSTATKDTYDALHMQALPPR

SEQ ID NO: 75 - DNA, 1455 bp, synthetic construct
  source 1..1455: mol_type = other DNA
atggccttaccagtgaccgccttgctcctgccgctggccttgctgctccacgccgccaggccggatattgtgataacccagtctccagcaatcatgtctgcatctccaggggagaaggtcaccatgacctgcagtgccagctcaagtgtaagttacatgcactggtaccagcagaagtcaggcacctcccccaaaagatggatttatgacacatccaaactggcttctggagtccctgctcgcttcagtggcagtgggtctgggacctcttactctctcacaatcagcagcatggaggctgaagatgctgccacttattactgccagcagtggagtagtaacccactcacgttcggtgctgggaccaagctggaaatcaaacgcggaggtgggggcagtggaggcggtggtagtggaggcggaggaagtcaggtccaactgcagcagtctggacctgagctggtgaagcctggcgcttcagtgaagatatcctgcaaggcttctggttactcattcactgactacaacatgaactgggtgaagcagagcaatggaaagagccttgagtggattggagtaattaatcctaactatggtactactagctacaatcagaagttcaagggcaaggccactataacagcagacacatcctccaacacagcctacctgcagctcagcagcctgacatctgaggactctgcagtctattactgtgcaaagggtgattacgacggggccgggtttgcttactggggccaagggactctggtcactgtctctgcgaccacgacgccagcgccgcgaccaccaacaccggcgcccaccatcgcgtcgcagcccctgtccctgcgcccagaggcgtgccggccagcggcggggggcgcagtgcacacgagggggctggacttcgcctgtgatatctacatctgggcgcccttggccgggacttgtggggtccttctcctgtcactggttatcaccctttactgcaaacggggcagaaagaaactcctgtatatattcaaacaaccatttatgagaccagtacaaactactcaagaggaagatggctgtagctgccgatttccagaagaagaagaaggaggatgtgaactgagagtgaagttcagcaggagcgcagacgcccccgcgtacaagcagggccagaaccagctctataacgagctcaatctaggacgaagagaggagtacgatgttttggacaagagacgtggccgggaccctgagatggggggaaagccgagaaggaagaaccctcaggaaggcctgtacaatgaactgcagaaagataagatggcggaggcctacagtgagattgggatgaaaggcgagcgccggaggggcaaggggcacgatggcctttaccagggtctcagtacagccaccaaggacacctacgacgcccttcacatgcaggccctgccccctcgc

SEQ ID NO: 76 - protein, 487 aa, synthetic construct
MALPVTALLLPLALLLHAARPDIVLTQSPAIMSTSPGEKVTMTCTASSSVSYMHWYQQKSGTSPKRWIYDTSKLASGVPARFSGSGSGTSYSLTISRMEAEDAATYYCQQWSSYPLTFGAGTKLEMKRGGGGSGGGGSGGGGSQVQLQQPGAELVKPGASVKLSCKASGYTFTSYWMHWVKQRPGQGLEWIGMIHPNSGGTNYNEKFKSKATLTVDKSSSTAYMQLSSLTSEDSAVYYCARYYYGNYVWYFDVWGTGTTVTVSATTTPAPRPPTPAPTIASQPLSLRPEACRPAAGGAVHTRGLDFACDIYIWAPLAGTCGVLLLSLVITLYCKRGRKKLLYIFKQPFMRPVQTTQEEDGCSCRFPEEEEGGCELRVKFSRSADAPAYKQGQNQLYNELNLGRREEYDVLDKRRGRDPEMGGKPRRKNPQEGLYNELQKDKMAEAYSEIGMKGERRRGKGHDGLYQGLSTATKDTYDALHMQALPPR

SEQ ID NO: 77 - DNA, 1461 bp, synthetic construct
  source 1..1461: mol_type = other DNA
atggccttaccagtgaccgccttgctcctgccgctggccttgctgctccacgccgccaggccggacattgttctcacccagtctccagcaatcatgtctacatctccgggggagaaggtcaccatgacctgcactgccagctcaagtgtaagttacatgcactggtaccagcagaagtcaggcacctcccccaaaagatggatttatgacacatccaaactggcttctggagtccctgctcgcttcagtggcagtgggtctgggacctcttactctctcacaatcagccgaatggaggctgaagatgctgccacttattactgccagcagtggagtagttacccactcacgttcggtgctgggaccaagctggaaatgaaacgcggaggtgggggcagtggaggcggtggtagtggaggcggaggaagtcaggtccaactgcagcagcctggggctgaactggtgaagcctggggcttcagtgaagctgtcctgcaaggcttctggctacaccttcaccagctactggatgcactgggtgaagcagaggcctggacaaggccttgagtggattggaatgattcatcctaatagtggtggtactaactacaatgagaagttcaagagcaaggccacactgactgtagacaaatcctccagcacagcctacatgcaactcagcagcctgacatctgaggactctgcggtctattactgtgcaagatactactatggtaactacgtgtggtacttcgatgtctggggcacagggaccacggtcaccgtctctgcgaccacgacgccagcgccgcgaccaccaacaccggcgcccaccatcgcgtcgcagcccctgtccctgcgcccagaggcgtgccggccagcggcggggggcgcagtgcacacgagggggctggacttcgcctgtgatatctacatctgggcgcccttggccgggacttgtggggtccttctcctgtcactggttatcaccctttactgcaaacggggcagaaagaaactcctgtatatattcaaacaaccatttatgagaccagtacaaactactcaagaggaagatggctgtagctgccgatttccagaagaagaagaaggaggatgtgaactgagagtgaagttcagcaggagcgcagacgcccccgcgtacaagcagggccagaaccagctctataacgagctcaatctaggacgaagagaggagtacgatgttttggacaagagacgtggccgggaccctgagatggggggaaagccgagaaggaagaaccctcaggaaggcctgtacaatgaactgcagaaagataagatggcggaggcctacagtgagattgggatgaaaggcgagcgccggaggggcaaggggcacgatggcctttaccagggtctcagtacagccaccaaggacacctacgacgcccttcacatgcaggccctgccccctcgc

SEQ ID NO: 78 - protein, 485 aa, synthetic construct
MALPVTALLLPLALLLHAARPEIVLTQSPATLSLSPGERATLSCSASSSVSYMHWYQQKPGQAPRLLIYDTSKLASGIPARFSGSGSGTDFTLTISSLEPEDFAVYYCQQWSSNPLTFGQGTKLEIKRGGGGSGGGGSGGGGSQVQLVQSGAEVKKPGASVKVSCKASGYTFTDYNMNWVRQAPGQGLEWMGVINPNYGTTSYNQKFKGRVTMTRDTSTSTVYMELSSLRSEDTAVYYCARGDYDGAGFAYWGQGTLVTVSSTTTPAPRPPTPAPTIASQPLSLRPEACRPAAGGAVHTRGLDFACDIYIWAPLAGTCGVLLLSLVITLYCKRGRKKLLYIFKQPFMRPVQTTQEEDGCSCRFPEEEEGGCELRVKFSRSADAPAYKQGQNQLYNELNLGRREEYDVLDKRRGRDPEMGGKPRRKNPQEGLYNELQKDKMAEAYSEIGMKGERRRGKGHDGLYQGLSTATKDTYDALHMQALPPR

SEQ ID NO: 79 - DNA, 1455 bp, synthetic construct
  source 1..1455: mol_type = other DNA
atggccttaccagtgaccgccttgctcctgccgctggccttgctgctccacgccgccaggccggaaattgtcttaacccagtctccagcaaccctttctttgtctccaggggagcgagcaaccctgagttgcagtgccagctcaagtgtaagttacatgcactggtaccagcagaagcctggccaagcgccccgccttctcatttatgacacatccaaactggcttctggaatacctgctcgcttcagtggcagtgggtctgggaccgactttactctcacaatcagcagcttggagccagaagattttgccgtatattactgccagcagtggagtagtaacccactcacgttcggtcaggggaccaagctggaaatcaaacgcggaggtgggggcagtggaggcggtggtagtggaggcggaggaagtcaggtccaactggttcagtctggagctgaggtaaagaagcctggcgcttcagtgaaggtttcctgcaaggcttctggttacaccttcactgactacaacatgaactgggtgcgacaggctcccggacaaggacttgagtggatgggagtaattaatcctaactatggtactactagctacaatcagaagttcaagggcagggtgactatgacacgcgacacatccacctctacagtgtacatggagctcagcagcctgcgctctgaggacacggcagtctattactgtgcaagaggtgattacgacggggccgggtttgcttactggggccaagggactctggtcactgtctctagcaccacgacgccagcgccgcgaccaccaacaccggcgcccaccatcgcgtcgcagcccctgtccctgcgcccagaggcgtgccggccagcggcggggggcgcagtgcacacgagggggctggacttcgcctgtgatatctacatctgggcgcccttggccgggacttgtggggtccttctcctgtcactggttatcaccctttactgcaaacggggcagaaagaaactcctgtatatattcaaacaaccatttatgagaccagtacaaactactcaagaggaagatggctgtagctgccgatttccagaagaagaagaaggaggatgtgaactgagagtgaagttcagcaggagcgcagacgcccccgcgtacaagcagggccagaaccagctctataacgagctcaatctaggacgaagagaggagtacgatgttttggacaagagacgtggccgggaccctgagatggggggaaagccgagaaggaagaaccctcaggaaggcctgtacaatgaactgcagaaagataagatggcggaggcctacagtgagattgggatgaaaggcgagcgccggaggggcaaggggcacgatggcctttaccagggtctcagtacagccaccaaggacacctacgacgcccttcacatgcaggccctgccccctcgc

SEQ ID NO: 80 - DNA, 33 bp, synthetic construct
  source 1..33: mol_type = other DNA
ggccgctagggccgaggttcdsctgcaacagty

SEQ ID NO: 81 - DNA, 33 bp, synthetic construct
  source 1..33: mol_type = other DNA
ggccgctagggcccaggtgcaamtgmagsagtc

SEQ ID NO: 82 - DNA, 33 bp, synthetic construct
  source 1..33: mol_type = other DNA
ggccgctagggccgavgtgmwgctggtggagtc

SEQ ID NO: 83 - DNA, 33 bp, synthetic construct
  source 1..33: mol_type = other DNA
ggccgctagggcccaggttaytctgaaagagtc

SEQ ID NO: 84 - DNA, 33 bp, synthetic construct
  source 1..33: mol_type = other DNA
ggccgctagggccgakgtgcagcttcagsagtc

SEQ ID NO: 85 - DNA, 33 bp, synthetic construct
  source 1..33: mol_type = other DNA
ggccgctagggcccagatccagttsgygcagtc

SEQ ID NO: 86 - DNA, 33 bp, synthetic construct
  source 1..33: mol_type = other DNA
ggccgctagggcccagrtccaactgcagcagyc

SEQ ID NO: 87 - DNA, 33 bp, synthetic construct
  source 1..33: mol_type = other DNA
ggccgctagggccgaggtgmagctasttgagwc

SEQ ID NO: 88 - DNA, 33 bp, synthetic construct
  source 1..33: mol_type = other DNA
ggccgctagggccgaagtgaagmttgaggagtc

SEQ ID NO: 89 - DNA, 33 bp, synthetic construct
  source 1..33: mol_type = other DNA
ggccgctagggccgatgtgaacctggaagtgtc

SEQ ID NO: 90 - DNA, 33 bp, synthetic construct
  source 1..33: mol_type = other DNA
ggccgctagggcccagatkcagcttmaggagtc

SEQ ID NO: 91 - DNA, 33 bp, synthetic construct
  source 1..33: mol_type = other DNA
ggccgctagggcccaggcttatctgcagcagtc

SEQ ID NO: 92 - DNA, 33 bp, synthetic construct
  source 1..33: mol_type = other DNA
ggccgctagggcccaggttcacctacaacagtc

SEQ ID NO: 93 - DNA, 33 bp, synthetic construct
  source 1..33: mol_type = other DNA
ggccgctagggcccaggtgcagcttgtagagac

SEQ ID NO: 94 - DNA, 33 bp, synthetic construct
  source 1..33: mol_type = other DNA
ggccgctagggccgargtgmagctgktggagac

SEQ ID NO: 95 - DNA, 20 bp, synthetic construct
  source 1..20: mol_type = other DNA
cgaggagacggtgacmgtgg

SEQ ID NO: 96 - DNA, 20 bp, synthetic construct
  source 1..20: mol_type = other DNA
cgcagagacagtgaccagag

SEQ ID NO: 97 - DNA, 20 bp, synthetic construct
  source 1..20: mol_type = other DNA
cgaggagactgtgagastgg

SEQ ID NO: 98 - DNA, 41 bp, synthetic construct
  source 1..41: mol_type = other DNA
ccackgtcaccgtctcctcggcctccaccaagggcccatcg

SEQ ID NO: 99 - DNA, 41 bp, synthetic construct
  source 1..41: mol_type = other DNA
ctctggtcactgtctctgcggcctccaccaagggcccatcg

SEQ ID NO: 100 - DNA, 41 bp, synthetic construct
  source 1..41: mol_type = other DNA
ccastctcacagtctcctcggcctccaccaagggcccatcg

SEQ ID NO: 101 - DNA, 30 bp, synthetic construct
  source 1..30: mol_type = other DNA
cgaattcagaacctcttggaactagcaagt

SEQ ID NO: 102 - DNA, 44 bp, synthetic construct
  source 1..44: mol_type = other DNA
gataaaagagaggccgctagggccgacawtgttctcacccagtc

SEQ ID NO: 103 - DNA, 44 bp, synthetic construct
  source 1..44: mol_type = other DNA
gataaaagagaggccgctagggccgacatccagatgacacagwc

SEQ ID NO: 104 - DNA, 44 bp, synthetic construct
  source 1..44: mol_type = other DNA
gataaaagagaggccgctagggccgatrttgtgatgacccagwc

SEQ ID NO: 105 - DNA, 44 bp, synthetic construct
  source 1..44: mol_type = other DNA
gataaaagagaggccgctagggccgacattstgmtgacccagtc

SEQ ID NO: 106 - DNA, 44 bp, synthetic construct
  source 1..44: mol_type = other DNA
gataaaagagaggccgctagggccgatgttgtgvtgacccaaac

SEQ ID NO: 107 - DNA, 44 bp, synthetic construct
  source 1..44: mol_type = other DNA
gataaaagagaggccgctagggccgacacaactgtgacccagtc

SEQ ID NO: 108 - DNA, 44 bp, synthetic construct
  source 1..44: mol_type = other DNA
gataaaagagaggccgctagggccgayattktgctcactcagtc

SEQ ID NO: 109 - DNA, 44 bp, synthetic construct
  source 1..44: mol_type = other DNA
gataaaagagaggccgctagggccgatattgtgatracccaggm

SEQ ID NO: 110 - DNA, 44 bp, synthetic construct
  source 1..44: mol_type = other DNA
gataaaagagaggccgctagggccgacattgtaatgacccaatc

SEQ ID NO: 111 - DNA, 44 bp, synthetic construct
  source 1..44: mol_type = other DNA
gataaaagagaggccgctagggccgacattgtgatgwcacagtc

SEQ ID NO: 112 - DNA, 44 bp, synthetic construct
  source 1..44: mol_type = other DNA
gataaaagagaggccgctagggccgatrtccagatgamccagtc

SEQ ID NO: 113 - DNA, 44 bp, synthetic construct
  source 1..44: mol_type = other DNA
gataaaagagaggccgctagggccgatggagaaacaacacaggc

SEQ ID NO: 114 - DNA, 43 bp, synthetic construct
  source 1..43: mol_type = other DNA
acagatggtgcagccaccgtacggcgtttbatttccagcttgg

SEQ ID NO: 115 - DNA, 43 bp, synthetic construct
  source 1..43: mol_type = other DNA
acagatggtgcagccaccgtacggcgttttatttccaattttg

SEQ ID NO: 116 - DNA, 23 bp, synthetic construct
  source 1..23: mol_type = other DNA
cgtacggtggctgcaccatctgt

SEQ ID NO: 117 - DNA, 31 bp, synthetic construct
  source 1..31: mol_type = other DNA
aattacatgactcgagctacttgtcatcgtc

SEQ ID NO: 118 - DNA, 26 bp, synthetic construct
  source 1..26: mol_type = other DNA
ccagcattgctgctaaagaagaaggg

SEQ ID NO: 119 - DNA, 30 bp, synthetic construct; identical to SEQ ID NO: 101
  source 1..30: mol_type = other DNA

SEQ ID NO: 120 - DNA, 27 bp, synthetic construct
  source 1..27: mol_type = other DNA
atgactcgagctacttgtcatcgtcgt

SEQ ID NO: 121 - DNA, 32 bp, synthetic construct
  source 1..32: mol_type = other DNA
cactatccaacagcacaaataacgggttatct

SEQ ID NO: 122 - DNA, 20 bp, synthetic construct
  source 1..20: mol_type = other DNA
ggaggagggtgccaggggga

SEQ ID NO: 123 - DNA, 32 bp, synthetic construct
  source 1..32: mol_type = other DNA
tgtactttggcctctctgggatagaagttatt